European Patent Application EP 4 725 965 A1, published April 15, 2026. Title: 抗BDCA2抗体. Applicant: 三生国健药业（上海）股份有限公司. The sequence listing filed with the application follows.

SEQUENCE LISTING (32 sequences)

SEQ ID NO: 1 - protein, 169 aa, synthetic construct
NFMYSKTVKRLSKLREYQQYHPSLTCVMEGKDIEDWSCCPTPWTSFQSSCYFISTGMQSWTKSQKNCSVMGADLVVINTREEQDFIIQNLKRNSSYFLGLSDPGGRRHWQWVDQTPYNENVTFWHSGEPNNLDERCAIINFRSSEEWGWNDIHCHVPQKSICKMKKIYI

SEQ ID NO: 2 - DNA, 354 bp, synthetic construct
  source 1..354: mol_type = other DNA
caggtgcaactacagcagcctggggctgacctggtgaagcctggggcctcagtgatgatgtcctgcaaggcttctggatacacatttaccagttacattattcactgggtaaaacagacacctggacagggcctggaatggattggaactatttatccaggaaatggtgatacttcctacaatcagaaattcaaaggcaaggccacattgactgcagacaaatcctccagcacagcctacatgcagctcagcagcctgacatctgaggactctgcggtctattactgtgcaagaatgggggataacgaatactttgactactggggccaaggaaccactctcacagtctcctca

SEQ ID NO: 3 - protein, 118 aa, synthetic construct
QVQLQQPGADLVKPGASVMMSCKASGYTFTSYIIHWVKQTPGQGLEWIGTIYPGNGDTSYNQKFKGKATLTADKSSSTAYMQLSSLTSEDSAVYYCARMGDNEYFDYWGQGTTLTVSS

SEQ ID NO: 4 - DNA, 321 bp, synthetic construct
  source 1..321: mol_type = other DNA
gacatccagatgactcagtctccagcctccctatctgcatctgtgggagaaactgtcaccatcacatgtcgagcaagtggaaatattcacaattatttagcatggtatcagcagaaacagggaaaatctcctcagctcctggtctatgatgcagaaaccttagcagatggtgtgccatcaaggttcagtggcagtggatccggaacacaatattctctcaatatcaacagcctgcagcctgaagattttgggagtttttactgtcaacatttttggagtactccgtacacgttcggaggggggaccaagctggaaataaaa

SEQ ID NO: 5 - protein, 107 aa, synthetic construct
DIQMTQSPASLSASVGETVTITCRASGNIHNYLAWYQQKQGKSPQLLVYDAETLADGVPSRFSGSGSGTQYSLNINSLQPEDFGSFYCQHFWSTPYTFGGGTKLEIK

SEQ ID NO: 6 - protein, 5 aa, synthetic construct
SYIIH

SEQ ID NO: 7 - protein, 17 aa, synthetic construct
TIYPGNGDTSYNQKFKG

SEQ ID NO: 8 - protein, 9 aa, synthetic construct
MGDNEYFDY

SEQ ID NO: 9 - protein, 11 aa, synthetic construct
RASGNIHNYLA

SEQ ID NO: 10 - protein, 7 aa, synthetic construct
DAETLAD

SEQ ID NO: 11 - protein, 9 aa, synthetic construct
QHFWSTPYT

SEQ ID NO: 12 - protein, 118 aa, synthetic construct
QVQLVQSGAEVKKPGASVKVSCKASGYTFTSYIIHWVRQAPGQGLEWMGTIYPGNGDTSYNQKFKGRVTMTRDTSTSTVYMELSSLRSEDTAVYYCARMGDNEYFDYWGQGTLVTVSS

SEQ ID NO: 13 - protein, 107 aa, synthetic construct
DIQMTQSPSSLSASVGDRVTITCRASGNIHNYLAWYQQKPGKAPKLLLYDAETLADGVPSRFSGSGSGTDYTLTISSLQPEDFATYYCQHFWSTPYTFGGGTKVEIK

SEQ ID NO: 14 - protein, 5 aa, synthetic construct
SYLIH

SEQ ID NO: 15 - protein, 17 aa, synthetic construct
TIYPGGGDTSYNQKFKG

SEQ ID NO: 16 - protein, 17 aa, synthetic construct
TIYPGAGDTSYNQKFKG

SEQ ID NO: 17 - protein, 17 aa, synthetic construct
TIYPGSGDTSYNQKFKG

SEQ ID NO: 18 - protein, 17 aa, synthetic construct
TIYPGRGDTSYNQKFKG

SEQ ID NO: 19 - protein, 7 aa, synthetic construct
DAETLAI

SEQ ID NO: 20 - protein, 7 aa, synthetic construct
DAETLAE

SEQ ID NO: 21 - protein, 118 aa, synthetic construct
QVQLVQSGAEVKKPGASVKVSCKASGYTFTSYLIHWVRQAPGQGLEWMGTIYPGNGDTSYNQKFKGRVTMTRDTSTSTVYMELSSLRSEDTAVYYCARMGDNEYFDYWGQGTLVTVSS

SEQ ID NO: 22 - protein, 118 aa, synthetic construct
QVQLVQSGAEVKKPGASVKVSCKASGYTFTSYLIHWVRQAPGQGLEWMGTIYPGGGDTSYNQKFKGRVTMTRDTSTSTVYMELSSLRSEDTAVYYCARMGDNEYFDYWGQGTLVTVSS

SEQ ID NO: 23 - protein, 118 aa, synthetic construct
QVQLVQSGAEVKKPGASVKVSCKASGYTFTSYLIHWVRQAPGQGLEWMGTIYPGRGDTSYNQKFKGRVTMTRDTSTSTVYMELSSLRSEDTAVYYCARMGDNEYFDYWGQGTLVTVSS

SEQ ID NO: 24 - protein, 118 aa, synthetic construct
QVQLVQSGAEVKKPGASVKVSCKASGYTFTSYIIHWVRQAPGQGLEWMGTIYPGGGDTSYNQKFKGRVTMTRDTSTSTVYMELSSLRSEDTAVYYCARMGDNEYFDYWGQGTLVTVSS

SEQ ID NO: 25 - protein, 118 aa, synthetic construct
QVQLVQSGAEVKKPGASVKVSCKASGYTFTSYIIHWVRQAPGQGLEWMGTIYPGRGDTSYNQKFKGRVTMTRDTSTSTVYMELSSLRSEDTAVYYCARMGDNEYFDYWGQGTLVTVSS

SEQ ID NO: 26 - protein, 107 aa, synthetic construct
DIQMTQSPSSLSASVGDRVTITCRASGNIHNYLAWYQQKPGKAPKLLLYDAETLAIGVPSRFSGSGSGTDYTLTISSLQPEDFATYYCQHFWSTPYTFGGGTKVEIK

SEQ ID NO: 27 - protein, 107 aa, synthetic construct
DIQMTQSPSSLSASVGDRVTITCRASGNIHNYLAWYQQKPGKAPKLLLYDAETLAEGVPSRFSGSGSGTDYTLTISSLQPEDFATYYCQHFWSTPYTFGGGTKVEIK

SEQ ID NO: 28 - protein, 448 aa, synthetic construct
QVQLVQSGAEVKKPGASVKVSCKASGYTFTSYLIHWVRQAPGQGLEWMGTIYPGGGDTSYNQKFKGRVTMTRDTSTSTVYMELSSLRSEDTAVYYCARMGDNEYFDYWGQGTLVTVSSASTKGPSVFPLAPSSKSTSGGTAALGCLVKDYFPEPVTVSWNSGALTSGVHTFPAVLQSSGLYSLSSVVTVPSSSLGTQTYICNVNHKPSNTKVDKKVEPKSCDKTHTCPPCPAPELLAGPDVFLFPPKPKDTLMISRTPEVTCVVVDVSHEDPEVKFNWYVDGVEVHNAKTKPREEQYNSTYRVVSVLTVLHQDWLNGKEYKCKVSNKALPAPEEKTISKAKGQPREPQVYTLPPSREEMTKNQVSLTCLVKGFYPSDIAVEWESNGQPENNYKTTPPVLDSDGSFFLYSKLTVDKSRWQQGNVFSCSVLHEALHSHYTQKSLSLSPGK

SEQ ID NO: 29 - protein, 448 aa, synthetic construct
QVQLVQSGAEVKKPGASVKVSCKASGYTFTSYIIHWVRQAPGQGLEWMGTIYPGGGDTSYNQKFKGRVTMTRDTSTSTVYMELSSLRSEDTAVYYCARMGDNEYFDYWGQGTLVTVSSASTKGPSVFPLAPSSKSTSGGTAALGCLVKDYFPEPVTVSWNSGALTSGVHTFPAVLQSSGLYSLSSVVTVPSSSLGTQTYICNVNHKPSNTKVDKKVEPKSCDKTHTCPPCPAPELLAGPDVFLFPPKPKDTLMISRTPEVTCVVVDVSHEDPEVKFNWYVDGVEVHNAKTKPREEQYNSTYRVVSVLTVLHQDWLNGKEYKCKVSNKALPAPEEKTISKAKGQPREPQVYTLPPSREEMTKNQVSLTCLVKGFYPSDIAVEWESNGQPENNYKTTPPVLDSDGSFFLYSKLTVDKSRWQQGNVFSCSVLHEALHSHYTQKSLSLSPGK

SEQ ID NO: 30 - protein, 5 aa, synthetic construct
  source 1..5: note = X= I or L
SYXIH

SEQ ID NO: 31 - protein, 17 aa, synthetic construct
  source 1..17: note = X=N or G or A or S or R
TIYPGXGDTSYNQKFKG

SEQ ID NO: 32 - protein, 7 aa, synthetic construct
  source 1..7: note = X=D or I or E
DAETLAX